European Patent Application EP 4 316 505 A1, published February 7, 2024. Title: Intranasal administration of NGF for the treatment of sensorineural hearing loss. Applicant: Dompé farmaceutici SpA. The sequence listing filed with the application follows.

SEQUENCE LISTING (6 sequences)

SEQ ID NO: 1 - protein, 118 aa, Homo sapiens
SSSHPIFHRGEFSVCDSVSVWVGDKTTATDIKGKEVMVLGEVNINNSVFKQYFFETKCRDPNPVDSGCRGIDSKHWNSYCTTTHTFVKALTMDGKQAAWRFIRIDTACVCVLSRKAVR

SEQ ID NO: 2 - protein, 120 aa, Homo sapiens
SSSHPIFHRGEFSVCDSVSVWVGDKTTATDIKGKEVMVLGEVNINNSVFKQYFFETKCRDPNPVDSGCRGIDSKHWNSYCTTTHTFVKALTMDGKQAAWRFIRIDTACVCVLSRKAVRRA

SEQ ID NO: 3 - protein, 118 aa, Homo sapiens
SSSHPIFHRGEFSVCDSVSVWVGDKTTATDIKGKEVMVLGEVNINNSVFKQYFFETKCRDPNPVDSGCRGIDSKHWNSYCTTTHTFVKALTMDGKQAAWEFIRIDTACVCVLSRKAVR

SEQ ID NO: 4 - protein, 120 aa, Homo sapiens
SSSHPIFHRGEFSVCDSVSVWVGDKTTATDIKGKEVMVLGEVNINNSVFKQYFFETKCRDPNPVDSGCRGIDSKHWNSYCTTTHTFVKALTMDGKQAAWEFIRIDTACVCVLSRKAVRRA

SEQ ID NO: 5 - protein, 118 aa, Homo sapiens
SSSHPIFHRGEFSVCDSVSVWVGDKTTATDIKGKEVMVLGEVNINNSVFKQYFFETKCRDSNPVDSGCRGIDSKHWNSYCTTTHTFVKALTMDGKQAAWEFIRIDTACVCVLSRKAVR

SEQ ID NO: 6 - protein, 120 aa, Homo sapiens
SSSHPIFHRGEFSVCDSVSVWVGDKTTATDIKGKEVMVLGEVNINNSVFKQYFFETKCRDSNPVDSGCRGIDSKHWNSYCTTTHTFVKALTMDGKQAAWEFIRIDTACVCVLSRKAVRRA